European Patent Application EP 4 682 168 A1, published January 21, 2026. Title: ANTI-LIV-1 ANTIBODY AND ANTI-LIV-1 ANTIBODY-DRUG CONJUGATE, AND PHARMACEUTICAL USE THEREOF. Applicant: BioRay Pharmaceutical Co., Ltd. Application EP. The sequence listing filed with the application follows.

SEQUENCE LISTING (34 sequences)

SEQ ID NO: 1 - protein, 120 aa, synthetic construct
EVQLVQSGAEVKKPGATVKISCKASGLNIEDYYMHWVQQAPGKGLEWMGWIDPENGDTEYAEKFQGRVTITADTSTNTAYMELSSLRSEDTAVYYCTVHNAHYGTWFAYWGQGTTVTVSS

SEQ ID NO: 2 - protein, 112 aa, synthetic construct
DIVMTQTPLSLSVTPGQPASISCRSSQTLVRSDGNTYLEWYLQKPGQSPQLLIYRVSNRFSGVPDRFSGSGSGTDFTLKISRVEAEDVGVYYCFQGSHVPYTFGGGTKLEIK

SEQ ID NO: 3 - protein, 116 aa, synthetic construct
EVQLQQSGAELVRSGASVKLSCTASGFNIKDYYMHWVKQRPEQGLEWIGWIDPENGDTEYAPKFQGKATLTADTSSNTAYLLLSSLTSEDTAVYYCKRRFYSMDYWGQGTSVTVSS

SEQ ID NO: 4 - protein, 112 aa, synthetic construct
DVLMTQTPLSLPVSLGDQASISCRSSQSIVHSNGNTYLEWYLQKPGQSPKLLIYKVSNRFSGVPDRFSGSGSGTDFTLKISRVEAEDLGVYYCFQGSHVPLTFGAGTKLELK

SEQ ID NO: 5 - protein, 118 aa, synthetic construct
DVQLQESGPGLVKPSQSLSLTCTVTGYSITSDYAWNWIRQFPGNKLEWMGYITYSGSTSYNPSLKSRISITRDTSKNQFFLQLNSVTTEDTATYYCAREGRLRPFAYWGQGTLVTVSA

SEQ ID NO: 6 - protein, 112 aa, synthetic construct
NIMMTQSPSSLAVSAGEKVTMSCKSSQSVLYSSNQKNYLAWYQQKPGQSPKLLIYWASTRESGVPDRFTGSGSGTDFTLTISSVQAEDLAVYYCHQYLSSWTFGGGTKLEIK

SEQ ID NO: 7 - protein, 5 aa, synthetic construct
DYYMH

SEQ ID NO: 8 - protein, 17 aa, synthetic construct
WIDPENGDTEYAEKFQG

SEQ ID NO: 9 - protein, 11 aa, synthetic construct
HNAHYGTWFAY

SEQ ID NO: 10 - protein, 16 aa, synthetic construct
RSSQTLVRSDGNTYLE

SEQ ID NO: 11 - protein, 7 aa, synthetic construct
RVSNRFS

SEQ ID NO: 12 - protein, 9 aa, synthetic construct
FQGSHVPYT

SEQ ID NO: 13 - protein, 5 aa, synthetic construct
DYYMH

SEQ ID NO: 14 - protein, 17 aa, synthetic construct
WIDPENGDTEYAPKFQG

SEQ ID NO: 15 - protein, 7 aa, synthetic construct
RFYSMDY

SEQ ID NO: 16 - protein, 16 aa, synthetic construct
RSSQSIVHSNGNTYLE

SEQ ID NO: 17 - protein, 7 aa, synthetic construct
KVSNRFS

SEQ ID NO: 18 - protein, 9 aa, synthetic construct
FQGSHVPLT

SEQ ID NO: 19 - protein, 6 aa, synthetic construct
SDYAWN

SEQ ID NO: 20 - protein, 16 aa, synthetic construct
YITYSGSTSYNPSLKS

SEQ ID NO: 21 - protein, 9 aa, synthetic construct
EGRLRPFAY

SEQ ID NO: 22 - protein, 17 aa, synthetic construct
KSSQSVLYSSNQKNYLA

SEQ ID NO: 23 - protein, 7 aa, synthetic construct
WASTRES

SEQ ID NO: 24 - protein, 8 aa, synthetic construct
HQYLSSWT

SEQ ID NO: 25 - protein, 755 aa, synthetic construct
MARKLSVILILTFALSVTNPLHELKAAAFPQTTEKISPNWESGINVDLAISTRQYHLQQLFYRYGENNSLSVEGFRKLLQNIGIDKIKRIHIHHDHDHHSDHEHHSDHERHSDHEHHSEHEHHSDHDHHSHHNHAASGKNKRKALCPDHDSDSSGKDPRNSQGKGAHRPEHASGRRNVKDSVSASEVTSTVYNTVSEGTHFLETIETPRPGKLFPKDVSSSTPPSVTSKSRVSRLAGRKTNESVSEPRKGFMYSRNTNENPQECFNASKLLTSHGMGIQVPLNATEFNYLCPAIINQIDARSCLIHTSEKKAEIPPKTYSLQIAWVGGFIAISIISFLSLLGVILVPLMNRVFFKFLLSFLVALAVGTLSGDAFLHLLPHSHASHHHSHSHEEPAMEMKRGPLFSHLSSQNIEESAYFDSTWKGLTALGGLYFMFLVEHVLTLIKQFKDKKKKNQKKPENDDDVEIKKQLSKYESQLSTNEEKVDTDDRTEGYLRADSQEPSHFDSQQPAVLEEEEVMIAHAHPQEVYNEYVPRGCKNKCHSHFHDTLGQSDDLIHHHHDYHHILHHHHHQNHHPHSHSQRYSREELKDAGVATLAWMVIMGDGLHNFSDGLAIGAAFTEGLSSGLSTSVAVFCHELPHELGDFAVLLKAGMTVKQAVLYNALSAMLAYLGMATGIFIGHYAENVSMWIFALTAGLFMYVALVDMVPEMLHNDASDHGCSRWGYFFLQNAGMLLGFGIMLLISIFEHKIVFRINF

SEQ ID NO: 26 - protein, 330 aa, synthetic construct [sequence omitted]

SEQ ID NO: 27 - protein, 107 aa, synthetic construct [sequence omitted]

SEQ ID NO: 28 - protein, 120 aa, synthetic construct
EVQLQQSGAELVRSGASVKVSCKASGLNIEDYYMHWVKQRPEQGLEWIGWIDPENGDTEYGPKFQGKATMTADTSSNTAYLQLSSLTSGDTAVYYCTVHNAHYGTWFAYWGQGTLVTVSS

SEQ ID NO: 29 - protein, 112 aa, synthetic construct
DVLMTQTPLSLPVSLGDQASISCRSSQTLVRSDGNTYLEWYLQKPGQSPKLLIYRVSNRFSGVPDRFSGSGSGTDFTLRISRVEAEDLGLYYCFQGSHVPYTFGGGTKLEIK

SEQ ID NO: 30 - protein, 219 aa, synthetic construct
DIVMTQTPLSLSVTPGQPASISCRSSQTLVRSDGNTYLEWYLQKPGQSPQLLIYRVSNRFSGVPDRFSGSGSGTDFTLKISRVEAEDVGVYYCFQGSHVPYTFGGGTKLEIKRTVAAPSVFIFPPSDEQLKSGTASVVCLLNNFYPREAKVQWKVDNALQSGNSQESVTEQDSKDSTYSLSSTLTLSKADYEKHKVYACEVTHQGLSSPVTKSFNRGEC

SEQ ID NO: 31 - protein, 450 aa, synthetic construct
EVQLVQSGAEVKKPGATVKISCKASGLNIEDYYMHWVQQAPGKGLEWMGWIDPENGDTEYAEKFQGRVTITADTSTNTAYMELSSLRSEDTAVYYCTVHNAHYGTWFAYWGQGTTVTVSSASTKGPSVFPLAPSSKSTSGGTAALGCLVKDYFPEPVTVSWNSGALTSGVHTFPAVLQSSGLYSLSSVVTVPSSSLGTQTYICNVNHKPSNTKVDKKVEPKSCDKTHTCPPCPAPELLGGPSVFLFPPKPKDTLMISRTPEVTCVVVDVSHEDPEVKFNWYVDGVEVHNAKTKPREEQYNSTYRVVSVLTVLHQDWLNGKEYKCKVSNKALPAPIEKTISKAKGQPREPQVYTLPPSRDELTKNQVSLTCLVKGFYPSDIAVEWESNGQPENNYKTTPPVLDSDGSFFLYSKLTVDKSRWQQGNVFSCSVMHEALHNHYTQKSLSLSPGK

SEQ ID NO: 32 - protein, 120 aa, synthetic construct
EVQLVQSGAEVKKPGATVKISCKASGLNIEDYYMHWVQQAPGKGLEWMGWIDPENGDTEYAEKFQGRVTITADTSTDTAYMELSSLRSEDTAVYYCTVHNAHYGTWFAYWGQGTTVTVSS

SEQ ID NO: 33 - protein, 450 aa, synthetic construct
QVQLVQSGAEVKKPGASVKVSCKASGLTIEDYYMHWVRQAPGQGLEWMGWIDPENGDTEYGPKFQGRVTMTRDTSINTAYMELSRLRSDDTAVYYCAVHNAHYGTWFAYWGQGTLVTVSSASTKGPSVFPLAPSSKSTSGGTAALGCLVKDYFPEPVTVSWNSGALTSGVHTFPAVLQSSGLYSLSSVVTVPSSSLGTQTYICNVNHKPSNTKVDKKVEPKSCDKTHTCPPCPAPELLGGPSVFLFPPKPKDTLMISRTPEVTCVVVDVSHEDPEVKFNWYVDGVEVHNAKTKPREEQYNSTYRVVSVLTVLHQDWLNGKEYKCKVSNKALPAPIEKTISKAKGQPREPQVYTLPPSRDELTKNQVSLTCLVKGFYPSDIAVEWESNGQPENNYKTTPPVLDSDGSFFLYSKLTVDKSRWQQGNVFSCSVMHEALHNHYTQKSLSLSPGK

SEQ ID NO: 34 - protein, 220 aa, synthetic construct
DVVMTQSPLSLPVTLGQPASISCRSSQSLLHSSGNTYLEWYQQRPGQSPRPLIYKISTRFSGVPDRFSGSGSGTDFTLKISRVEAEDVGVYYCFQGSHVPYTFGGGTKVEIKRRTVAAPSVFIFPPSDEQLKSGTASVVCLLNNFYPREAKVQWKVDNALQSGNSQESVTEQDSKDSTYSLSSTLTLSKADYEKHKVYACEVTHQGLSSPVTKSFNRGEC